European Patent Application EP 4 786 589 A1, published August 5, 2026. Title: non-natural 3' untranslated region and use thereof. Applicant: HANMI PHARM. CO., LTD. The sequence listing filed with the application follows.

SEQUENCE LISTING (35 sequences)

SEQ ID NO: 1 - RNA, 178 nt, synthetic construct
  source 1..178: mol_type = other RNA
accaccaagacaaaaaccacgaatttacgccaaaagtggagtaaggaggtgcgtcccttacgcaacacgacagccgggatctaacaatagggttaatggactggttgagataaggggcattaaaaccaaacggtctacacataaaacgaatgaaaacttcctaaaggatcgacggtgg

SEQ ID NO: 2 - RNA, 178 nt, synthetic construct
  source 1..178: mol_type = other RNA
cataccataaaaccaaacatatacccgaggtccttcggcattgggaggatgatacgcaagaagcatgattccccaccagaccgaatgcaggtttaagtgaggggtgcaaacttgtgtcactaaccattattatgaagaaaaaaacagccaaaaaaagagccacaaggcggcgcggtat

SEQ ID NO: 3 - RNA, 178 nt, synthetic construct
  source 1..178: mol_type = other RNA
gccgctaaataaacgaacacgtacctacgctttgacaggagtgggcaagtgggaaggttaccggaactacgaggaccaccaggcaagtattggttagtcactcttccaactaatcttaataaaacgagacatcgaaaaaaaaaaaaggcaaaaacaagtccagaaggagccagggtgg

SEQ ID NO: 4 - RNA, 178 nt, synthetic construct
  source 1..178: mol_type = other RNA
agagtaaaattaatatacggtatagaactcaccattgtgcgttctacctcgaggtgtcatgacgacagtgtcccatatcaacccgagaagttggaaatgcggagtcgaacgtgacgccaataaggccaaaaggtaaataatgaaacgtacaaccgaatgccaaaaggctacgctgctc

SEQ ID NO: 5 - RNA, 178 nt, synthetic construct
  source 1..178: mol_type = other RNA
gtacatgctacaaaccatgcggaacctacaagacactttatgggtaaagcaacaaacccacttgtaaagttaccacaccggtcccatctgccggccgtgagtatatgatctgggtttataatctcgaaatatcgcgaaacaatatgcccttagaataagcacccatgcgggcaatgta

SEQ ID NO: 6 - RNA, 158 nt, synthetic construct
  source 1..158: mol_type = other RNA
tagtaatacagcatagtgacgcaaaattattacgagtacaattaatcagtacttgttggtcatagcaaccaaagtggaaaaagttgtgttattaaaaccccaaaacaaacgattgtttcaatggggtcataactaatgtaacgttaggtaattatccg

SEQ ID NO: 7 - RNA, 158 nt, synthetic construct
  source 1..158: mol_type = other RNA
tctttatgagaattactcattctgatttttaacatagcattttttttctgttgtgtagatgggccaaaggacattccataacttttcataaggacaaacgattaccgacggattggtactagttgttaattaacatctgggggatgtaaacatttttt

SEQ ID NO: 8 - RNA, 158 nt, synthetic construct
  source 1..158: mol_type = other RNA
aacacagaaaactaccactatacttctatttagaaagcacttattaattgctttttgttagtgaaacatgcaaggcacccatgttttctgtgttaaccaagccagttgatattagctgtatgcttggattctatacataaaatgtatttaagcagctc

SEQ ID NO: 9 - RNA, 178 nt, Homo sapiens
  source 1..178: mol_type = mRNA
ccacacccccattcccccactccagataaagcttcagttatatctcacgtgtctggagttctttgccaagagggagaggctgaaatccccagccgcctcacctgcagctcagctccatcctacttgaaacctcacctgttcccaccgcattttctcctggcgttcgcctgctagtgtg

SEQ ID NO: 10 - RNA, 158 nt, Homo sapiens
  source 1..158: mol_type = mRNA
gtgtgtggaggacaccctgaaccccccgctttcaaacaagttttcaaattgtttgaggtcaggatttctcaaactgattcctttctttgcatatgagtatttgaaaataaatattttcccagaatataaataaatcatcacatgattattttaactat

SEQ ID NO: 11 - protein, 393 aa, Homo sapiens [sequence omitted]

SEQ ID NO: 12 - DNA, 17 bp, synthetic construct
  source 1..17: mol_type = other DNA
taatacgactcactata

SEQ ID NO: 13 - DNA, 61 bp, synthetic construct
  source 1..61: mol_type = other DNA
agtgctccccatccaactaaactgtccctctgtccgaactaaactgcactgtcccagcacc

SEQ ID NO: 14 - DNA, 1179 bp, Homo sapiens
  source 1..1179: mol_type = genomic DNA
atggaagaacctcagtccgatccgagcgtcgagcctcccctgtcacaggaaactttcagtgacctgtggaaactgctgcccgagaataatgtactttcgcctctgcctagccaagcaatggatgatctgatgctgtctccagatgacatcgaacagtggtttacagaggatccagggcccgatgaggcaccacgaatgccagaggcggccccacctgttgcacccgcacctgcggctccaacacccgcagcccccgcccccgctccaagctggcctctcagtagttccgtgccatcacagaagacctatcaaggcagctacggatttcgcctcggatttctccattcaggcactgccaagtccgtgacttgtacgtacagccccgctctgaacaaaatgttctgtcagttggcgaagacatgtcctgtccagctttgggtagattctacccccccgccggggacacgggtgcgagccatggccatttataaacagtctcagcacatgaccgaggtcgtgcgcaggtgtcctcaccatgaacgatgctccgactccgacggcctggcccccccacagcacctgattcgcgtggaaggcaatcttcgtgtggagtacctcgatgatcggaacaccttcagacatagcgtggttgtgccttatgagccacccgaagttggaagcgactgtaccaccatccattacaactatatgtgcaacagtagctgcatgggtggcatgaatcggcggcctatcttgacaataatcactttagaggactcttccggaaacctgcttggcagaaattcattcgaggtccgtgtctgcgcctgcccgggcagggaccgcagaaccgaagaggagaatttacggaaaaagggggaaccccaccacgaactgccaccgggcagtaccaaaagggctctccctaataacacatcttcatcgccccagccaaagaagaaacccctcgacggagagtactttactctacaaattagggggagagaaagatttgagatgttccgcgaattgaacgaggccctggagttgaaagacgctcaagccggaaaggaaccaggtgggtctagggcccactcaagccatctgaagagtaagaaaggccagtccacttccaggcacaaaaagttaatgttcaagacggagggtcctgactctgac

SEQ ID NO: 15 - DNA, 158 bp, Homo sapiens
  source 1..158: mol_type = genomic DNA
gtgtgtggaggacaccctgaaccccccgctttcaaacaagttttcaaattgtttgaggtcaggatttctcaaactgattcctttctttgcatatgagtatttgaaaataaatattttcccagaatataaataaatcatcacatgattattttaactat

SEQ ID NO: 16 - DNA, 100 bp, synthetic construct
  source 1..100: mol_type = other DNA
aaaaaaaaaaaaaaaaaaaaaaaaaaaaaaaaaaaaaaaaaaaaaaaaaaaaaaaaaaaaaaaaaaaaaaaaaaaaaaaaaaaaaaaaaaaaaaaaaaaa

SEQ ID NO: 17 - RNA, 61 nt, Homo sapiens
  source 1..61: mol_type = other RNA
agtcctccccatcctctccctctgtccctctgtccctctgaccctgcactgtcccagcacc

SEQ ID NO: 18 - RNA, 1398 nt, synthetic construct
  source 1..1398: mol_type = other RNA
agtcctccccatcctctccctctgtccctctgtccctctgaccctgcactgtcccagcaccatggaagaacctcagtccgatccgagcgtcgagcctcccctgtcacaggaaactttcagtgacctgtggaaactgctgcccgagaataatgtactttcgcctctgcctagccaagcaatggatgatctgatgctgtctccagatgacatcgaacagtggtttacagaggatccagggcccgatgaggcaccacgaatgccagaggcggccccacctgttgcacccgcacctgcggctccaacacccgcagcccccgcccccgctccaagctggcctctcagtagttccgtgccatcacagaagacctatcaaggcagctacggatttcgcctcggatttctccattcaggcactgccaagtccgtgacttgtacgtacagccccgctctgaacaaaatgttctgtcagttggcgaagacatgtcctgtccagctttgggtagattctacccccccgccggggacacgggtgcgagccatggccatttataaacagtctcagcacatgaccgaggtcgtgcgcaggtgtcctcaccatgaacgatgctccgactccgacggcctggcccccccacagcacctgattcgcgtggaaggcaatcttcgtgtggagtacctcgatgatcggaacaccttcagacatagcgtggttgtgccttatgagccacccgaagttggaagcgactgtaccaccatccattacaactatatgtgcaacagtagctgcatgggtggcatgaatcggcggcctatcttgacaataatcactttagaggactcttccggaaacctgcttggcagaaattcattcgaggtccgtgtctgcgcctgcccgggcagggaccgcagaaccgaagaggagaatttacggaaaaagggggaaccccaccacgaactgccaccgggcagtaccaaaagggctctccctaataacacatcttcatcgccccagccaaagaagaaacccctcgacggagagtactttactctacaaattagggggagagaaagatttgagatgttccgcgaattgaacgaggccctggagttgaaagacgctcaagccggaaaggaaccaggtgggtctagggcccactcaagccatctgaagagtaagaaaggccagtccacttccaggcacaaaaagttaatgttcaagacggagggtcctgactctgacgtgtgtggaggacaccctgaaccccccgctttcaaacaagttttcaaattgtttgaggtcaggatttctcaaactgattcctttctttgcatatgagtatttgaaaataaatattttcccagaatataaataaatcatcacatgattattttaactat

SEQ ID NO: 19 - RNA, 1418 nt, synthetic construct
  source 1..1418: mol_type = other RNA
agtcctccccatcctctccctctgtccctctgtccctctgaccctgcactgtcccagcaccatggaagaacctcagtccgatccgagcgtcgagcctcccctgtcacaggaaactttcagtgacctgtggaaactgctgcccgagaataatgtactttcgcctctgcctagccaagcaatggatgatctgatgctgtctccagatgacatcgaacagtggtttacagaggatccagggcccgatgaggcaccacgaatgccagaggcggccccacctgttgcacccgcacctgcggctccaacacccgcagcccccgcccccgctccaagctggcctctcagtagttccgtgccatcacagaagacctatcaaggcagctacggatttcgcctcggatttctccattcaggcactgccaagtccgtgacttgtacgtacagccccgctctgaacaaaatgttctgtcagttggcgaagacatgtcctgtccagctttgggtagattctacccccccgccggggacacgggtgcgagccatggccatttataaacagtctcagcacatgaccgaggtcgtgcgcaggtgtcctcaccatgaacgatgctccgactccgacggcctggcccccccacagcacctgattcgcgtggaaggcaatcttcgtgtggagtacctcgatgatcggaacaccttcagacatagcgtggttgtgccttatgagccacccgaagttggaagcgactgtaccaccatccattacaactatatgtgcaacagtagctgcatgggtggcatgaatcggcggcctatcttgacaataatcactttagaggactcttccggaaacctgcttggcagaaattcattcgaggtccgtgtctgcgcctgcccgggcagggaccgcagaaccgaagaggagaatttacggaaaaagggggaaccccaccacgaactgccaccgggcagtaccaaaagggctctccctaataacacatcttcatcgccccagccaaagaagaaacccctcgacggagagtactttactctacaaattagggggagagaaagatttgagatgttccgcgaattgaacgaggccctggagttgaaagacgctcaagccggaaaggaaccaggtgggtctagggcccactcaagccatctgaagagtaagaaaggccagtccacttccaggcacaaaaagttaatgttcaagacggagggtcctgactctgacaccaccaagacaaaaaccacgaatttacgccaaaagtggagtaaggaggtgcgtcccttacgcaacacgacagccgggatctaacaatagggttaatggactggttgagataaggggcattaaaaccaaacggtctacacataaaacgaatgaaaacttcctaaaggatcgacggtgg

SEQ ID NO: 20 - RNA, 1418 nt, synthetic construct
  source 1..1418: mol_type = other RNA
agtcctccccatcctctccctctgtccctctgtccctctgaccctgcactgtcccagcaccatggaagaacctcagtccgatccgagcgtcgagcctcccctgtcacaggaaactttcagtgacctgtggaaactgctgcccgagaataatgtactttcgcctctgcctagccaagcaatggatgatctgatgctgtctccagatgacatcgaacagtggtttacagaggatccagggcccgatgaggcaccacgaatgccagaggcggccccacctgttgcacccgcacctgcggctccaacacccgcagcccccgcccccgctccaagctggcctctcagtagttccgtgccatcacagaagacctatcaaggcagctacggatttcgcctcggatttctccattcaggcactgccaagtccgtgacttgtacgtacagccccgctctgaacaaaatgttctgtcagttggcgaagacatgtcctgtccagctttgggtagattctacccccccgccggggacacgggtgcgagccatggccatttataaacagtctcagcacatgaccgaggtcgtgcgcaggtgtcctcaccatgaacgatgctccgactccgacggcctggcccccccacagcacctgattcgcgtggaaggcaatcttcgtgtggagtacctcgatgatcggaacaccttcagacatagcgtggttgtgccttatgagccacccgaagttggaagcgactgtaccaccatccattacaactatatgtgcaacagtagctgcatgggtggcatgaatcggcggcctatcttgacaataatcactttagaggactcttccggaaacctgcttggcagaaattcattcgaggtccgtgtctgcgcctgcccgggcagggaccgcagaaccgaagaggagaatttacggaaaaagggggaaccccaccacgaactgccaccgggcagtaccaaaagggctctccctaataacacatcttcatcgccccagccaaagaagaaacccctcgacggagagtactttactctacaaattagggggagagaaagatttgagatgttccgcgaattgaacgaggccctggagttgaaagacgctcaagccggaaaggaaccaggtgggtctagggcccactcaagccatctgaagagtaagaaaggccagtccacttccaggcacaaaaagttaatgttcaagacggagggtcctgactctgaccataccataaaaccaaacatatacccgaggtccttcggcattgggaggatgatacgcaagaagcatgattccccaccagaccgaatgcaggtttaagtgaggggtgcaaacttgtgtcactaaccattattatgaagaaaaaaacagccaaaaaaagagccacaaggcggcgcggtat

SEQ ID NO: 21 - RNA, 1418 nt, synthetic construct
  source 1..1418: mol_type = other RNA
agtcctccccatcctctccctctgtccctctgtccctctgaccctgcactgtcccagcaccatggaagaacctcagtccgatccgagcgtcgagcctcccctgtcacaggaaactttcagtgacctgtggaaactgctgcccgagaataatgtactttcgcctctgcctagccaagcaatggatgatctgatgctgtctccagatgacatcgaacagtggtttacagaggatccagggcccgatgaggcaccacgaatgccagaggcggccccacctgttgcacccgcacctgcggctccaacacccgcagcccccgcccccgctccaagctggcctctcagtagttccgtgccatcacagaagacctatcaaggcagctacggatttcgcctcggatttctccattcaggcactgccaagtccgtgacttgtacgtacagccccgctctgaacaaaatgttctgtcagttggcgaagacatgtcctgtccagctttgggtagattctacccccccgccggggacacgggtgcgagccatggccatttataaacagtctcagcacatgaccgaggtcgtgcgcaggtgtcctcaccatgaacgatgctccgactccgacggcctggcccccccacagcacctgattcgcgtggaaggcaatcttcgtgtggagtacctcgatgatcggaacaccttcagacatagcgtggttgtgccttatgagccacccgaagttggaagcgactgtaccaccatccattacaactatatgtgcaacagtagctgcatgggtggcatgaatcggcggcctatcttgacaataatcactttagaggactcttccggaaacctgcttggcagaaattcattcgaggtccgtgtctgcgcctgcccgggcagggaccgcagaaccgaagaggagaatttacggaaaaagggggaaccccaccacgaactgccaccgggcagtaccaaaagggctctccctaataacacatcttcatcgccccagccaaagaagaaacccctcgacggagagtactttactctacaaattagggggagagaaagatttgagatgttccgcgaattgaacgaggccctggagttgaaagacgctcaagccggaaaggaaccaggtgggtctagggcccactcaagccatctgaagagtaagaaaggccagtccacttccaggcacaaaaagttaatgttcaagacggagggtcctgactctgacgccgctaaataaacgaacacgtacctacgctttgacaggagtgggcaagtgggaaggttaccggaactacgaggaccaccaggcaagtattggttagtcactcttccaactaatcttaataaaacgagacatcgaaaaaaaaaaaaggcaaaaacaagtccagaaggagccagggtgg

SEQ ID NO: 22 - RNA, 1418 nt, synthetic construct
  source 1..1418: mol_type = other RNA
agtcctccccatcctctccctctgtccctctgtccctctgaccctgcactgtcccagcaccatggaagaacctcagtccgatccgagcgtcgagcctcccctgtcacaggaaactttcagtgacctgtggaaactgctgcccgagaataatgtactttcgcctctgcctagccaagcaatggatgatctgatgctgtctccagatgacatcgaacagtggtttacagaggatccagggcccgatgaggcaccacgaatgccagaggcggccccacctgttgcacccgcacctgcggctccaacacccgcagcccccgcccccgctccaagctggcctctcagtagttccgtgccatcacagaagacctatcaaggcagctacggatttcgcctcggatttctccattcaggcactgccaagtccgtgacttgtacgtacagccccgctctgaacaaaatgttctgtcagttggcgaagacatgtcctgtccagctttgggtagattctacccccccgccggggacacgggtgcgagccatggccatttataaacagtctcagcacatgaccgaggtcgtgcgcaggtgtcctcaccatgaacgatgctccgactccgacggcctggcccccccacagcacctgattcgcgtggaaggcaatcttcgtgtggagtacctcgatgatcggaacaccttcagacatagcgtggttgtgccttatgagccacccgaagttggaagcgactgtaccaccatccattacaactatatgtgcaacagtagctgcatgggtggcatgaatcggcggcctatcttgacaataatcactttagaggactcttccggaaacctgcttggcagaaattcattcgaggtccgtgtctgcgcctgcccgggcagggaccgcagaaccgaagaggagaatttacggaaaaagggggaaccccaccacgaactgccaccgggcagtaccaaaagggctctccctaataacacatcttcatcgccccagccaaagaagaaacccctcgacggagagtactttactctacaaattagggggagagaaagatttgagatgttccgcgaattgaacgaggccctggagttgaaagacgctcaagccggaaaggaaccaggtgggtctagggcccactcaagccatctgaagagtaagaaaggccagtccacttccaggcacaaaaagttaatgttcaagacggagggtcctgactctgacagagtaaaattaatatacggtatagaactcaccattgtgcgttctacctcgaggtgtcatgacgacagtgtcccatatcaacccgagaagttggaaatgcggagtcgaacgtgacgccaataaggccaaaaggtaaataatgaaacgtacaaccgaatgccaaaaggctacgctgctc

SEQ ID NO: 23 - RNA, 1418 nt, synthetic construct
  source 1..1418: mol_type = other RNA
agtcctccccatcctctccctctgtccctctgtccctctgaccctgcactgtcccagcaccatggaagaacctcagtccgatccgagcgtcgagcctcccctgtcacaggaaactttcagtgacctgtggaaactgctgcccgagaataatgtactttcgcctctgcctagccaagcaatggatgatctgatgctgtctccagatgacatcgaacagtggtttacagaggatccagggcccgatgaggcaccacgaatgccagaggcggccccacctgttgcacccgcacctgcggctccaacacccgcagcccccgcccccgctccaagctggcctctcagtagttccgtgccatcacagaagacctatcaaggcagctacggatttcgcctcggatttctccattcaggcactgccaagtccgtgacttgtacgtacagccccgctctgaacaaaatgttctgtcagttggcgaagacatgtcctgtccagctttgggtagattctacccccccgccggggacacgggtgcgagccatggccatttataaacagtctcagcacatgaccgaggtcgtgcgcaggtgtcctcaccatgaacgatgctccgactccgacggcctggcccccccacagcacctgattcgcgtggaaggcaatcttcgtgtggagtacctcgatgatcggaacaccttcagacatagcgtggttgtgccttatgagccacccgaagttggaagcgactgtaccaccatccattacaactatatgtgcaacagtagctgcatgggtggcatgaatcggcggcctatcttgacaataatcactttagaggactcttccggaaacctgcttggcagaaattcattcgaggtccgtgtctgcgcctgcccgggcagggaccgcagaaccgaagaggagaatttacggaaaaagggggaaccccaccacgaactgccaccgggcagtaccaaaagggctctccctaataacacatcttcatcgccccagccaaagaagaaacccctcgacggagagtactttactctacaaattagggggagagaaagatttgagatgttccgcgaattgaacgaggccctggagttgaaagacgctcaagccggaaaggaaccaggtgggtctagggcccactcaagccatctgaagagtaagaaaggccagtccacttccaggcacaaaaagttaatgttcaagacggagggtcctgactctgacgtacatgctacaaaccatgcggaacctacaagacactttatgggtaaagcaacaaacccacttgtaaagttaccacaccggtcccatctgccggccgtgagtatatgatctgggtttataatctcgaaatatcgcgaaacaatatgcccttagaataagcacccatgcgggcaatgta

SEQ ID NO: 24 - RNA, 1398 nt, synthetic construct
  source 1..1398: mol_type = other RNA
agtcctccccatcctctccctctgtccctctgtccctctgaccctgcactgtcccagcaccatggaagaacctcagtccgatccgagcgtcgagcctcccctgtcacaggaaactttcagtgacctgtggaaactgctgcccgagaataatgtactttcgcctctgcctagccaagcaatggatgatctgatgctgtctccagatgacatcgaacagtggtttacagaggatccagggcccgatgaggcaccacgaatgccagaggcggccccacctgttgcacccgcacctgcggctccaacacccgcagcccccgcccccgctccaagctggcctctcagtagttccgtgccatcacagaagacctatcaaggcagctacggatttcgcctcggatttctccattcaggcactgccaagtccgtgacttgtacgtacagccccgctctgaacaaaatgttctgtcagttggcgaagacatgtcctgtccagctttgggtagattctacccccccgccggggacacgggtgcgagccatggccatttataaacagtctcagcacatgaccgaggtcgtgcgcaggtgtcctcaccatgaacgatgctccgactccgacggcctggcccccccacagcacctgattcgcgtggaaggcaatcttcgtgtggagtacctcgatgatcggaacaccttcagacatagcgtggttgtgccttatgagccacccgaagttggaagcgactgtaccaccatccattacaactatatgtgcaacagtagctgcatgggtggcatgaatcggcggcctatcttgacaataatcactttagaggactcttccggaaacctgcttggcagaaattcattcgaggtccgtgtctgcgcctgcccgggcagggaccgcagaaccgaagaggagaatttacggaaaaagggggaaccccaccacgaactgccaccgggcagtaccaaaagggctctccctaataacacatcttcatcgccccagccaaagaagaaacccctcgacggagagtactttactctacaaattagggggagagaaagatttgagatgttccgcgaattgaacgaggccctggagttgaaagacgctcaagccggaaaggaaccaggtgggtctagggcccactcaagccatctgaagagtaagaaaggccagtccacttccaggcacaaaaagttaatgttcaagacggagggtcctgactctgactagtaatacagcatagtgacgcaaaattattacgagtacaattaatcagtacttgttggtcatagcaaccaaagtggaaaaagttgtgttattaaaaccccaaaacaaacgattgtttcaatggggtcataactaatgtaacgttaggtaattatccg

SEQ ID NO: 25 - RNA, 1398 nt, synthetic construct
  source 1..1398: mol_type = other RNA
agtcctccccatcctctccctctgtccctctgtccctctgaccctgcactgtcccagcaccatggaagaacctcagtccgatccgagcgtcgagcctcccctgtcacaggaaactttcagtgacctgtggaaactgctgcccgagaataatgtactttcgcctctgcctagccaagcaatggatgatctgatgctgtctccagatgacatcgaacagtggtttacagaggatccagggcccgatgaggcaccacgaatgccagaggcggccccacctgttgcacccgcacctgcggctccaacacccgcagcccccgcccccgctccaagctggcctctcagtagttccgtgccatcacagaagacctatcaaggcagctacggatttcgcctcggatttctccattcaggcactgccaagtccgtgacttgtacgtacagccccgctctgaacaaaatgttctgtcagttggcgaagacatgtcctgtccagctttgggtagattctacccccccgccggggacacgggtgcgagccatggccatttataaacagtctcagcacatgaccgaggtcgtgcgcaggtgtcctcaccatgaacgatgctccgactccgacggcctggcccccccacagcacctgattcgcgtggaaggcaatcttcgtgtggagtacctcgatgatcggaacaccttcagacatagcgtggttgtgccttatgagccacccgaagttggaagcgactgtaccaccatccattacaactatatgtgcaacagtagctgcatgggtggcatgaatcggcggcctatcttgacaataatcactttagaggactcttccggaaacctgcttggcagaaattcattcgaggtccgtgtctgcgcctgcccgggcagggaccgcagaaccgaagaggagaatttacggaaaaagggggaaccccaccacgaactgccaccgggcagtaccaaaagggctctccctaataacacatcttcatcgccccagccaaagaagaaacccctcgacggagagtactttactctacaaattagggggagagaaagatttgagatgttccgcgaattgaacgaggccctggagttgaaagacgctcaagccggaaaggaaccaggtgggtctagggcccactcaagccatctgaagagtaagaaaggccagtccacttccaggcacaaaaagttaatgttcaagacggagggtcctgactctgactctttatgagaattactcattctgatttttaacatagcattttttttctgttgtgtagatgggccaaaggacattccataacttttcataaggacaaacgattaccgacggattggtactagttgttaattaacatctgggggatgtaaacatttttt

SEQ ID NO: 26 - RNA, 1398 nt, synthetic construct
  source 1..1398: mol_type = other RNA
agtcctccccatcctctccctctgtccctctgtccctctgaccctgcactgtcccagcaccatggaagaacctcagtccgatccgagcgtcgagcctcccctgtcacaggaaactttcagtgacctgtggaaactgctgcccgagaataatgtactttcgcctctgcctagccaagcaatggatgatctgatgctgtctccagatgacatcgaacagtggtttacagaggatccagggcccgatgaggcaccacgaatgccagaggcggccccacctgttgcacccgcacctgcggctccaacacccgcagcccccgcccccgctccaagctggcctctcagtagttccgtgccatcacagaagacctatcaaggcagctacggatttcgcctcggatttctccattcaggcactgccaagtccgtgacttgtacgtacagccccgctctgaacaaaatgttctgtcagttggcgaagacatgtcctgtccagctttgggtagattctacccccccgccggggacacgggtgcgagccatggccatttataaacagtctcagcacatgaccgaggtcgtgcgcaggtgtcctcaccatgaacgatgctccgactccgacggcctggcccccccacagcacctgattcgcgtggaaggcaatcttcgtgtggagtacctcgatgatcggaacaccttcagacatagcgtggttgtgccttatgagccacccgaagttggaagcgactgtaccaccatccattacaactatatgtgcaacagtagctgcatgggtggcatgaatcggcggcctatcttgacaataatcactttagaggactcttccggaaacctgcttggcagaaattcattcgaggtccgtgtctgcgcctgcccgggcagggaccgcagaaccgaagaggagaatttacggaaaaagggggaaccccaccacgaactgccaccgggcagtaccaaaagggctctccctaataacacatcttcatcgccccagccaaagaagaaacccctcgacggagagtactttactctacaaattagggggagagaaagatttgagatgttccgcgaattgaacgaggccctggagttgaaagacgctcaagccggaaaggaaccaggtgggtctagggcccactcaagccatctgaagagtaagaaaggccagtccacttccaggcacaaaaagttaatgttcaagacggagggtcctgactctgacaacacagaaaactaccactatacttctatttagaaagcacttattaattgctttttgttagtgaaacatgcaaggcacccatgttttctgtgttaaccaagccagttgatattagctgtatgcttggattctatacataaaatgtatttaagcagctc

SEQ ID NO: 27 - RNA, 1498 nt, synthetic construct
  source 1..1498: mol_type = other RNA
agtcctccccatcctctccctctgtccctctgtccctctgaccctgcactgtcccagcaccatggaagaacctcagtccgatccgagcgtcgagcctcccctgtcacaggaaactttcagtgacctgtggaaactgctgcccgagaataatgtactttcgcctctgcctagccaagcaatggatgatctgatgctgtctccagatgacatcgaacagtggtttacagaggatccagggcccgatgaggcaccacgaatgccagaggcggccccacctgttgcacccgcacctgcggctccaacacccgcagcccccgcccccgctccaagctggcctctcagtagttccgtgccatcacagaagacctatcaaggcagctacggatttcgcctcggatttctccattcaggcactgccaagtccgtgacttgtacgtacagccccgctctgaacaaaatgttctgtcagttggcgaagacatgtcctgtccagctttgggtagattctacccccccgccggggacacgggtgcgagccatggccatttataaacagtctcagcacatgaccgaggtcgtgcgcaggtgtcctcaccatgaacgatgctccgactccgacggcctggcccccccacagcacctgattcgcgtggaaggcaatcttcgtgtggagtacctcgatgatcggaacaccttcagacatagcgtggttgtgccttatgagccacccgaagttggaagcgactgtaccaccatccattacaactatatgtgcaacagtagctgcatgggtggcatgaatcggcggcctatcttgacaataatcactttagaggactcttccggaaacctgcttggcagaaattcattcgaggtccgtgtctgcgcctgcccgggcagggaccgcagaaccgaagaggagaatttacggaaaaagggggaaccccaccacgaactgccaccgggcagtaccaaaagggctctccctaataacacatcttcatcgccccagccaaagaagaaacccctcgacggagagtactttactctacaaattagggggagagaaagatttgagatgttccgcgaattgaacgaggccctggagttgaaagacgctcaagccggaaaggaaccaggtgggtctagggcccactcaagccatctgaagagtaagaaaggccagtccacttccaggcacaaaaagttaatgttcaagacggagggtcctgactctgacgtgtgtggaggacaccctgaaccccccgctttcaaacaagttttcaaattgtttgaggtcaggatttctcaaactgattcctttctttgcatatgagtatttgaaaataaatattttcccagaatataaataaatcatcacatgattattttaactataaaaaaaaaaaaaaaaaaaaaaaaaaaaaaaaaaaaaaaaaaaaaaaaaaaaaaaaaaaaaaaaaaaaaaaaaaaaaaaaaaaaaaaaaaaaaaaaaaaa

SEQ ID NO: 28 - RNA, 1518 nt, synthetic construct
  source 1..1518: mol_type = other RNA
agtcctccccatcctctccctctgtccctctgtccctctgaccctgcactgtcccagcaccatggaagaacctcagtccgatccgagcgtcgagcctcccctgtcacaggaaactttcagtgacctgtggaaactgctgcccgagaataatgtactttcgcctctgcctagccaagcaatggatgatctgatgctgtctccagatgacatcgaacagtggtttacagaggatccagggcccgatgaggcaccacgaatgccagaggcggccccacctgttgcacccgcacctgcggctccaacacccgcagcccccgcccccgctccaagctggcctctcagtagttccgtgccatcacagaagacctatcaaggcagctacggatttcgcctcggatttctccattcaggcactgccaagtccgtgacttgtacgtacagccccgctctgaacaaaatgttctgtcagttggcgaagacatgtcctgtccagctttgggtagattctacccccccgccggggacacgggtgcgagccatggccatttataaacagtctcagcacatgaccgaggtcgtgcgcaggtgtcctcaccatgaacgatgctccgactccgacggcctggcccccccacagcacctgattcgcgtggaaggcaatcttcgtgtggagtacctcgatgatcggaacaccttcagacatagcgtggttgtgccttatgagccacccgaagttggaagcgactgtaccaccatccattacaactatatgtgcaacagtagctgcatgggtggcatgaatcggcggcctatcttgacaataatcactttagaggactcttccggaaacctgcttggcagaaattcattcgaggtccgtgtctgcgcctgcccgggcagggaccgcagaaccgaagaggagaatttacggaaaaagggggaaccccaccacgaactgccaccgggcagtaccaaaagggctctccctaataacacatcttcatcgccccagccaaagaagaaacccctcgacggagagtactttactctacaaattagggggagagaaagatttgagatgttccgcgaattgaacgaggccctggagttgaaagacgctcaagccggaaaggaaccaggtgggtctagggcccactcaagccatctgaagagtaagaaaggccagtccacttccaggcacaaaaagttaatgttcaagacggagggtcctgactctgacaccaccaagacaaaaaccacgaatttacgccaaaagtggagtaaggaggtgcgtcccttacgcaacacgacagccgggatctaacaatagggttaatggactggttgagataaggggcattaaaaccaaacggtctacacataaaacgaatgaaaacttcctaaaggatcgacggtggaaaaaaaaaaaaaaaaaaaaaaaaaaaaaaaaaaaaaaaaaaaaaaaaaaaaaaaaaaaaaaaaaaaaaaaaaaaaaaaaaaaaaaaaaaaaaaaaaaaa

SEQ ID NO: 29 - RNA, 1518 nt, synthetic construct
  source 1..1518: mol_type = other RNA
agtcctccccatcctctccctctgtccctctgtccctctgaccctgcactgtcccagcaccatggaagaacctcagtccgatccgagcgtcgagcctcccctgtcacaggaaactttcagtgacctgtggaaactgctgcccgagaataatgtactttcgcctctgcctagccaagcaatggatgatctgatgctgtctccagatgacatcgaacagtggtttacagaggatccagggcccgatgaggcaccacgaatgccagaggcggccccacctgttgcacccgcacctgcggctccaacacccgcagcccccgcccccgctccaagctggcctctcagtagttccgtgccatcacagaagacctatcaaggcagctacggatttcgcctcggatttctccattcaggcactgccaagtccgtgacttgtacgtacagccccgctctgaacaaaatgttctgtcagttggcgaagacatgtcctgtccagctttgggtagattctacccccccgccggggacacgggtgcgagccatggccatttataaacagtctcagcacatgaccgaggtcgtgcgcaggtgtcctcaccatgaacgatgctccgactccgacggcctggcccccccacagcacctgattcgcgtggaaggcaatcttcgtgtggagtacctcgatgatcggaacaccttcagacatagcgtggttgtgccttatgagccacccgaagttggaagcgactgtaccaccatccattacaactatatgtgcaacagtagctgcatgggtggcatgaatcggcggcctatcttgacaataatcactttagaggactcttccggaaacctgcttggcagaaattcattcgaggtccgtgtctgcgcctgcccgggcagggaccgcagaaccgaagaggagaatttacggaaaaagggggaaccccaccacgaactgccaccgggcagtaccaaaagggctctccctaataacacatcttcatcgccccagccaaagaagaaacccctcgacggagagtactttactctacaaattagggggagagaaagatttgagatgttccgcgaattgaacgaggccctggagttgaaagacgctcaagccggaaaggaaccaggtgggtctagggcccactcaagccatctgaagagtaagaaaggccagtccacttccaggcacaaaaagttaatgttcaagacggagggtcctgactctgaccataccataaaaccaaacatatacccgaggtccttcggcattgggaggatgatacgcaagaagcatgattccccaccagaccgaatgcaggtttaagtgaggggtgcaaacttgtgtcactaaccattattatgaagaaaaaaacagccaaaaaaagagccacaaggcggcgcggtataaaaaaaaaaaaaaaaaaaaaaaaaaaaaaaaaaaaaaaaaaaaaaaaaaaaaaaaaaaaaaaaaaaaaaaaaaaaaaaaaaaaaaaaaaaaaaaaaaaa

SEQ ID NO: 30 - RNA, 1518 nt, synthetic construct
  source 1..1518: mol_type = other RNA
agtcctccccatcctctccctctgtccctctgtccctctgaccctgcactgtcccagcaccatggaagaacctcagtccgatccgagcgtcgagcctcccctgtcacaggaaactttcagtgacctgtggaaactgctgcccgagaataatgtactttcgcctctgcctagccaagcaatggatgatctgatgctgtctccagatgacatcgaacagtggtttacagaggatccagggcccgatgaggcaccacgaatgccagaggcggccccacctgttgcacccgcacctgcggctccaacacccgcagcccccgcccccgctccaagctggcctctcagtagttccgtgccatcacagaagacctatcaaggcagctacggatttcgcctcggatttctccattcaggcactgccaagtccgtgacttgtacgtacagccccgctctgaacaaaatgttctgtcagttggcgaagacatgtcctgtccagctttgggtagattctacccccccgccggggacacgggtgcgagccatggccatttataaacagtctcagcacatgaccgaggtcgtgcgcaggtgtcctcaccatgaacgatgctccgactccgacggcctggcccccccacagcacctgattcgcgtggaaggcaatcttcgtgtggagtacctcgatgatcggaacaccttcagacatagcgtggttgtgccttatgagccacccgaagttggaagcgactgtaccaccatccattacaactatatgtgcaacagtagctgcatgggtggcatgaatcggcggcctatcttgacaataatcactttagaggactcttccggaaacctgcttggcagaaattcattcgaggtccgtgtctgcgcctgcccgggcagggaccgcagaaccgaagaggagaatttacggaaaaagggggaaccccaccacgaactgccaccgggcagtaccaaaagggctctccctaataacacatcttcatcgccccagccaaagaagaaacccctcgacggagagtactttactctacaaattagggggagagaaagatttgagatgttccgcgaattgaacgaggccctggagttgaaagacgctcaagccggaaaggaaccaggtgggtctagggcccactcaagccatctgaagagtaagaaaggccagtccacttccaggcacaaaaagttaatgttcaagacggagggtcctgactctgacgccgctaaataaacgaacacgtacctacgctttgacaggagtgggcaagtgggaaggttaccggaactacgaggaccaccaggcaagtattggttagtcactcttccaactaatcttaataaaacgagacatcgaaaaaaaaaaaaggcaaaaacaagtccagaaggagccagggtggaaaaaaaaaaaaaaaaaaaaaaaaaaaaaaaaaaaaaaaaaaaaaaaaaaaaaaaaaaaaaaaaaaaaaaaaaaaaaaaaaaaaaaaaaaaaaaaaaaaa

SEQ ID NO: 31 - RNA, 1518 nt, synthetic construct
  source 1..1518: mol_type = other RNA
agtcctccccatcctctccctctgtccctctgtccctctgaccctgcactgtcccagcaccatggaagaacctcagtccgatccgagcgtcgagcctcccctgtcacaggaaactttcagtgacctgtggaaactgctgcccgagaataatgtactttcgcctctgcctagccaagcaatggatgatctgatgctgtctccagatgacatcgaacagtggtttacagaggatccagggcccgatgaggcaccacgaatgccagaggcggccccacctgttgcacccgcacctgcggctccaacacccgcagcccccgcccccgctccaagctggcctctcagtagttccgtgccatcacagaagacctatcaaggcagctacggatttcgcctcggatttctccattcaggcactgccaagtccgtgacttgtacgtacagccccgctctgaacaaaatgttctgtcagttggcgaagacatgtcctgtccagctttgggtagattctacccccccgccggggacacgggtgcgagccatggccatttataaacagtctcagcacatgaccgaggtcgtgcgcaggtgtcctcaccatgaacgatgctccgactccgacggcctggcccccccacagcacctgattcgcgtggaaggcaatcttcgtgtggagtacctcgatgatcggaacaccttcagacatagcgtggttgtgccttatgagccacccgaagttggaagcgactgtaccaccatccattacaactatatgtgcaacagtagctgcatgggtggcatgaatcggcggcctatcttgacaataatcactttagaggactcttccggaaacctgcttggcagaaattcattcgaggtccgtgtctgcgcctgcccgggcagggaccgcagaaccgaagaggagaatttacggaaaaagggggaaccccaccacgaactgccaccgggcagtaccaaaagggctctccctaataacacatcttcatcgccccagccaaagaagaaacccctcgacggagagtactttactctacaaattagggggagagaaagatttgagatgttccgcgaattgaacgaggccctggagttgaaagacgctcaagccggaaaggaaccaggtgggtctagggcccactcaagccatctgaagagtaagaaaggccagtccacttccaggcacaaaaagttaatgttcaagacggagggtcctgactctgacagagtaaaattaatatacggtatagaactcaccattgtgcgttctacctcgaggtgtcatgacgacagtgtcccatatcaacccgagaagttggaaatgcggagtcgaacgtgacgccaataaggccaaaaggtaaataatgaaacgtacaaccgaatgccaaaaggctacgctgctcaaaaaaaaaaaaaaaaaaaaaaaaaaaaaaaaaaaaaaaaaaaaaaaaaaaaaaaaaaaaaaaaaaaaaaaaaaaaaaaaaaaaaaaaaaaaaaaaaaaa

SEQ ID NO: 32 - RNA, 1518 nt, synthetic construct
  source 1..1518: mol_type = other RNA
agtcctccccatcctctccctctgtccctctgtccctctgaccctgcactgtcccagcaccatggaagaacctcagtccgatccgagcgtcgagcctcccctgtcacaggaaactttcagtgacctgtggaaactgctgcccgagaataatgtactttcgcctctgcctagccaagcaatggatgatctgatgctgtctccagatgacatcgaacagtggtttacagaggatccagggcccgatgaggcaccacgaatgccagaggcggccccacctgttgcacccgcacctgcggctccaacacccgcagcccccgcccccgctccaagctggcctctcagtagttccgtgccatcacagaagacctatcaaggcagctacggatttcgcctcggatttctccattcaggcactgccaagtccgtgacttgtacgtacagccccgctctgaacaaaatgttctgtcagttggcgaagacatgtcctgtccagctttgggtagattctacccccccgccggggacacgggtgcgagccatggccatttataaacagtctcagcacatgaccgaggtcgtgcgcaggtgtcctcaccatgaacgatgctccgactccgacggcctggcccccccacagcacctgattcgcgtggaaggcaatcttcgtgtggagtacctcgatgatcggaacaccttcagacatagcgtggttgtgccttatgagccacccgaagttggaagcgactgtaccaccatccattacaactatatgtgcaacagtagctgcatgggtggcatgaatcggcggcctatcttgacaataatcactttagaggactcttccggaaacctgcttggcagaaattcattcgaggtccgtgtctgcgcctgcccgggcagggaccgcagaaccgaagaggagaatttacggaaaaagggggaaccccaccacgaactgccaccgggcagtaccaaaagggctctccctaataacacatcttcatcgccccagccaaagaagaaacccctcgacggagagtactttactctacaaattagggggagagaaagatttgagatgttccgcgaattgaacgaggccctggagttgaaagacgctcaagccggaaaggaaccaggtgggtctagggcccactcaagccatctgaagagtaagaaaggccagtccacttccaggcacaaaaagttaatgttcaagacggagggtcctgactctgacgtacatgctacaaaccatgcggaacctacaagacactttatgggtaaagcaacaaacccacttgtaaagttaccacaccggtcccatctgccggccgtgagtatatgatctgggtttataatctcgaaatatcgcgaaacaatatgcccttagaataagcacccatgcgggcaatgtaaaaaaaaaaaaaaaaaaaaaaaaaaaaaaaaaaaaaaaaaaaaaaaaaaaaaaaaaaaaaaaaaaaaaaaaaaaaaaaaaaaaaaaaaaaaaaaaaaaaa

SEQ ID NO: 33 - RNA, 1498 nt, synthetic construct
  source 1..1498: mol_type = other RNA
agtcctccccatcctctccctctgtccctctgtccctctgaccctgcactgtcccagcaccatggaagaacctcagtccgatccgagcgtcgagcctcccctgtcacaggaaactttcagtgacctgtggaaactgctgcccgagaataatgtactttcgcctctgcctagccaagcaatggatgatctgatgctgtctccagatgacatcgaacagtggtttacagaggatccagggcccgatgaggcaccacgaatgccagaggcggccccacctgttgcacccgcacctgcggctccaacacccgcagcccccgcccccgctccaagctggcctctcagtagttccgtgccatcacagaagacctatcaaggcagctacggatttcgcctcggatttctccattcaggcactgccaagtccgtgacttgtacgtacagccccgctctgaacaaaatgttctgtcagttggcgaagacatgtcctgtccagctttgggtagattctacccccccgccggggacacgggtgcgagccatggccatttataaacagtctcagcacatgaccgaggtcgtgcgcaggtgtcctcaccatgaacgatgctccgactccgacggcctggcccccccacagcacctgattcgcgtggaaggcaatcttcgtgtggagtacctcgatgatcggaacaccttcagacatagcgtggttgtgccttatgagccacccgaagttggaagcgactgtaccaccatccattacaactatatgtgcaacagtagctgcatgggtggcatgaatcggcggcctatcttgacaataatcactttagaggactcttccggaaacctgcttggcagaaattcattcgaggtccgtgtctgcgcctgcccgggcagggaccgcagaaccgaagaggagaatttacggaaaaagggggaaccccaccacgaactgccaccgggcagtaccaaaagggctctccctaataacacatcttcatcgccccagccaaagaagaaacccctcgacggagagtactttactctacaaattagggggagagaaagatttgagatgttccgcgaattgaacgaggccctggagttgaaagacgctcaagccggaaaggaaccaggtgggtctagggcccactcaagccatctgaagagtaagaaaggccagtccacttccaggcacaaaaagttaatgttcaagacggagggtcctgactctgactagtaatacagcatagtgacgcaaaattattacgagtacaattaatcagtacttgttggtcatagcaaccaaagtggaaaaagttgtgttattaaaaccccaaaacaaacgattgtttcaatggggtcataactaatgtaacgttaggtaattatccgaaaaaaaaaaaaaaaaaaaaaaaaaaaaaaaaaaaaaaaaaaaaaaaaaaaaaaaaaaaaaaaaaaaaaaaaaaaaaaaaaaaaaaaaaaaaaaaaaaaa

SEQ ID NO: 34 - RNA, 1498 nt, synthetic construct
  source 1..1498: mol_type = other RNA
agtcctccccatcctctccctctgtccctctgtccctctgaccctgcactgtcccagcaccatggaagaacctcagtccgatccgagcgtcgagcctcccctgtcacaggaaactttcagtgacctgtggaaactgctgcccgagaataatgtactttcgcctctgcctagccaagcaatggatgatctgatgctgtctccagatgacatcgaacagtggtttacagaggatccagggcccgatgaggcaccacgaatgccagaggcggccccacctgttgcacccgcacctgcggctccaacacccgcagcccccgcccccgctccaagctggcctctcagtagttccgtgccatcacagaagacctatcaaggcagctacggatttcgcctcggatttctccattcaggcactgccaagtccgtgacttgtacgtacagccccgctctgaacaaaatgttctgtcagttggcgaagacatgtcctgtccagctttgggtagattctacccccccgccggggacacgggtgcgagccatggccatttataaacagtctcagcacatgaccgaggtcgtgcgcaggtgtcctcaccatgaacgatgctccgactccgacggcctggcccccccacagcacctgattcgcgtggaaggcaatcttcgtgtggagtacctcgatgatcggaacaccttcagacatagcgtggttgtgccttatgagccacccgaagttggaagcgactgtaccaccatccattacaactatatgtgcaacagtagctgcatgggtggcatgaatcggcggcctatcttgacaataatcactttagaggactcttccggaaacctgcttggcagaaattcattcgaggtccgtgtctgcgcctgcccgggcagggaccgcagaaccgaagaggagaatttacggaaaaagggggaaccccaccacgaactgccaccgggcagtaccaaaagggctctccctaataacacatcttcatcgccccagccaaagaagaaacccctcgacggagagtactttactctacaaattagggggagagaaagatttgagatgttccgcgaattgaacgaggccctggagttgaaagacgctcaagccggaaaggaaccaggtgggtctagggcccactcaagccatctgaagagtaagaaaggccagtccacttccaggcacaaaaagttaatgttcaagacggagggtcctgactctgactctttatgagaattactcattctgatttttaacatagcattttttttctgttgtgtagatgggccaaaggacattccataacttttcataaggacaaacgattaccgacggattggtactagttgttaattaacatctgggggatgtaaacattttttaaaaaaaaaaaaaaaaaaaaaaaaaaaaaaaaaaaaaaaaaaaaaaaaaaaaaaaaaaaaaaaaaaaaaaaaaaaaaaaaaaaaaaaaaaaaaaaaaaaa

SEQ ID NO: 35 - RNA, 1498 nt, synthetic construct
  source 1..1498: mol_type = other RNA
agtcctccccatcctctccctctgtccctctgtccctctgaccctgcactgtcccagcaccatggaagaacctcagtccgatccgagcgtcgagcctcccctgtcacaggaaactttcagtgacctgtggaaactgctgcccgagaataatgtactttcgcctctgcctagccaagcaatggatgatctgatgctgtctccagatgacatcgaacagtggtttacagaggatccagggcccgatgaggcaccacgaatgccagaggcggccccacctgttgcacccgcacctgcggctccaacacccgcagcccccgcccccgctccaagctggcctctcagtagttccgtgccatcacagaagacctatcaaggcagctacggatttcgcctcggatttctccattcaggcactgccaagtccgtgacttgtacgtacagccccgctctgaacaaaatgttctgtcagttggcgaagacatgtcctgtccagctttgggtagattctacccccccgccggggacacgggtgcgagccatggccatttataaacagtctcagcacatgaccgaggtcgtgcgcaggtgtcctcaccatgaacgatgctccgactccgacggcctggcccccccacagcacctgattcgcgtggaaggcaatcttcgtgtggagtacctcgatgatcggaacaccttcagacatagcgtggttgtgccttatgagccacccgaagttggaagcgactgtaccaccatccattacaactatatgtgcaacagtagctgcatgggtggcatgaatcggcggcctatcttgacaataatcactttagaggactcttccggaaacctgcttggcagaaattcattcgaggtccgtgtctgcgcctgcccgggcagggaccgcagaaccgaagaggagaatttacggaaaaagggggaaccccaccacgaactgccaccgggcagtaccaaaagggctctccctaataacacatcttcatcgccccagccaaagaagaaacccctcgacggagagtactttactctacaaattagggggagagaaagatttgagatgttccgcgaattgaacgaggccctggagttgaaagacgctcaagccggaaaggaaccaggtgggtctagggcccactcaagccatctgaagagtaagaaaggccagtccacttccaggcacaaaaagttaatgttcaagacggagggtcctgactctgacaacacagaaaactaccactatacttctatttagaaagcacttattaattgctttttgttagtgaaacatgcaaggcacccatgttttctgtgttaaccaagccagttgatattagctgtatgcttggattctatacataaaatgtatttaagcagctcaaaaaaaaaaaaaaaaaaaaaaaaaaaaaaaaaaaaaaaaaaaaaaaaaaaaaaaaaaaaaaaaaaaaaaaaaaaaaaaaaaaaaaaaaaaaaaaaaaaa